European Patent Specification EP 4 107 178 B1, published January 10, 2024. Title: AFFINITY LIGAND FOR THE SOLUBLE PART OF FIBROBLAST GROWTH FACTOR RECEPTOR 3 (sFGFR3). Applicant: Navigo Proteins GmbH. The sequence listing filed with the application follows.

SEQUENCE LISTING (48 sequences)

SEQ ID NO: 1 - protein, 58 aa, Artificial Sequence
  sFGFR3 binding protein 1 (204815 monomer)
IAAKFDHKQSTADTIILELPNLTEEQRNAFRQSLSDDPSVSKEVLYEAIWLNWSQAPK

SEQ ID NO: 2 - protein, 58 aa, Artificial Sequence
  sFGFR3 binding protein 2 (204783 monomer)
IAAKFDQHQSTADEIILKLPNLTEEQRNAFRQSLSDDTSVSREVLYEALWLNASQAPK

SEQ ID NO: 3 - protein, 58 aa, Artificial Sequence
  sFGFR3 binding protein 3 (206146 monomer)
IAAKFDYVQSMADAQILQLINLTEEQRNAFRQSLSDDPSVSMVVLYRADWLNEHQAPK

SEQ ID NO: 4 - protein, 58 aa, Artificial Sequence
  sFGFR3 binding protein 4 (206142 monomer)
IAAKFDYIQHMADDYILQLRNLTEEQRNAFRQSLSDDPSVSMVVLYRADWLNEHQAPK

SEQ ID NO: 5 - protein, 58 aa, Artificial Sequence
  sFGFR3 binding protein 5 (206141 monomer)
IAAKFDYIQEMADKHILMLHNLTEEQRNAFRQSLSDDPSVSMLVLYKAHWLNQSQAPK

SEQ ID NO: 6 - protein, 58 aa, Artificial Sequence
  sFGFR3 binding protein 6 (206137 monomer)
IAAKFDDIQMMADAQILILYNLTEEQRNAFRQSLSDDPSVSLVVLYKADWLNRHQAPK

SEQ ID NO: 7 - protein, 58 aa, Artificial Sequence
  sFGFR3 binding protein 7 (206136 monomer)
IAAKFDQIQAMADQYILHLMNLTEEQRNAFRQSLSDDPSVSMIVLYKADWLNDKQAPK

SEQ ID NO: 8 - protein, 58 aa, Artificial Sequence
  sFGFR3 binding protein 8 (206121 monomer)
IAAKFDEAQSAADSEILHLPNLTEYHRIQHRYWLVWDPSVSQFTLRDAQALNDWQAPK

SEQ ID NO: 9 - protein, 58 aa, Artificial Sequence
  sFGFR3 binding protein 9 (206113 monomer)
NAASEDWAQFSAMYEIDHLPNLTMRQAIWFIHSLYHDPSVSKEVLGEAQKLNDSQAPK

SEQ ID NO: 10 - protein, 58 aa, Artificial Sequence
  sFGFR3 binding protein  (consensus sequence for SEQs 1 - 7)
  Xaa (7)..(7): Xaa may be selected from any amino acid, preferably H, Q, Y, or D
  Xaa (8)..(8): Xaa may be selected from any amino acid, preferably H, K, V, or I
  Xaa (10)..(10): Xaa may be selected from any amino acid, preferably S, H, E, M, or A
  Xaa (11)..(11): Xaa may be selected from any amino acid, preferably T or M
  Xaa (14)..(14): Xaa may be selected from any amino acid, preferably T or E
  misc_feature (15)..(15): Xaa can be any naturally occurring amino acid
  Xaa (18)..(18): Xaa may be selected from any amino acid, preferably K or E
  Xaa (20)..(20): Xaa may be selected from any amino acid, preferably P, I, R, H, Y, or M
  Xaa (38)..(38): Xaa may be selected from any amino acid, preferably P or T
  Xaa (42)..(42): Xaa may be selected from any amino acid, preferably K, R, M, or L
  Xaa (43)..(43): Xaa may be selected from any amino acid, preferably E, V, L, or I
  Xaa (47)..(47): Xaa may be selected from any amino acid, preferably E, R, or K
  Xaa (49)..(49): Xaa may be selected from any amino acid, preferably I, L, D, or H
  Xaa (53)..(53): Xaa may be selected from any amino acid, preferably W, A, E, Q, R, or D
IAAKFDXXQXXADXXILXLXNLTEEQRNAFRQSLSDDXSVSXXVLYXAXWLNXSQAPK

SEQ ID NO: 11 - protein, 175 aa, Artificial Sequence
  sFGFR3 binding protein  (tetramer of SEQ ID NO: 1; CID206078)
IAAKFDHKQSTADTIILELPNLTEEQRNAFRQSLSDDPSVSKEVLYEAIWLNWSQAPKIAAKFDHKQSTADTIILELPNLTEEQRNAFRQSLSDDPSVSKEVLYEAIWLNWSQAPKIAAKFDHKQSTADTIILELPNLTEEQRNAFRQSLSDDPSVSKEVLYEAIWLNWSQAPKC

SEQ ID NO: 12 - protein, 174 aa, Artificial Sequence
  fusion protein CID204815 (SEQ ID NO: 1 with PAdelFc)
IAAKFDEAQSAADSEILHLPNLTEEQRNAFRQSLSDDPSVSLEVLGEAQKLNDSQAPKIAAKFDHKQSTADTIILELPNLTEEQRNAFRQSLSDDPSVSKEVLYEAIWLNWSQAPKIAAKFDEAQSAADSEILHLPNLTEEQRNAFRQSLSDDPSVSLEVLGEAQKLNDSQAPK

SEQ ID NO: 13 - protein, 174 aa, Artificial Sequence
  fusion protein CID204783 (SEQ ID NO: 2 with PAdelFc)
IAAKFDEAQSAADSEILHLPNLTEEQRNAFRQSLSDDPSVSLEVLGEAQKLNDSQAPKIAAKFDQHQSTADEIILKLPNLTEEQRNAFRQSLSDDTSVSREVLYEALWLNASQAPKIAAKFDEAQSAADSEILHLPNLTEEQRNAFRQSLSDDPSVSLEVLGEAQKLNDSQAPK

SEQ ID NO: 14 - protein, 185 aa, Artificial Sequence
  fusion protein CID204815 (SEQ ID NO: 1 with PAdelFc; Streptag, Cys)
IAAKFDEAQSAADSEILHLPNLTEEQRNAFRQSLSDDPSVSLEVLGEAQKLNDSQAPKIAAKFDHKQSTADTIILELPNLTEEQRNAFRQSLSDDPSVSKEVLYEAIWLNWSQAPKIAAKFDEAQSAADSEILHLPNLTEEQRNAFRQSLSDDPSVSLEVLGEAQKLNDSQAPKCSAWSHPQFEK

SEQ ID NO: 15 - protein, 185 aa, Artificial Sequence
  fusion protein CID204783 (SEQ ID NO: 2 with PAdelFc; Streptag, Cys)
IAAKFDEAQSAADSEILHLPNLTEEQRNAFRQSLSDDPSVSLEVLGEAQKLNDSQAPKIAAKFDQHQSTADEIILKLPNLTEEQRNAFRQSLSDDTSVSREVLYEALWLNASQAPKIAAKFDEAQSAADSEILHLPNLTEEQRNAFRQSLSDDPSVSLEVLGEAQKLNDSQAPKCSAWSHPQFEK

SEQ ID NO: 16 - protein, 174 aa, Artificial Sequence
  fusion protein CID206113 (SEQ ID NO: 9 with PAdelFc)
IAAKFDEAQSAADSEILHLPNLTEEQRNAFRQSLSDDPSVSLEVLGEAQKLNDSQAPKNAASEDWAQFSAMYEIDHLPNLTMRQAIWFIHSLYHDPSVSKEVLGEAQKLNDSQAPKIAAKFDEAQSAADSEILHLPNLTEEQRNAFRQSLSDDPSVSLEVLGEAQKLNDSQAPK

SEQ ID NO: 17 - protein, 174 aa, Artificial Sequence
  fusion protein CID206121 (SEQ ID NO: 8 with PAdelFc)
IAAKFDEAQSAADSEILHLPNLTEEQRNAFRQSLSDDPSVSLEVLGEAQKLNDSQAPKIAAKFDEAQSAADSEILHLPNLTEYHRIQHRYWLVWDPSVSQFTLRDAQALNDWQAPKIAAKFDEAQSAADSEILHLPNLTEEQRNAFRQSLSDDPSVSLEVLGEAQKLNDSQAPK

SEQ ID NO: 18 - protein, 174 aa, Artificial Sequence
  fusion protein CID206136 (SEQ ID NO: 7 with PAdelFc)
IAAKFDEAQSAADSEILHLPNLTEEQRNAFRQSLSDDPSVSLEVLGEAQKLNDSQAPKIAAKFDQIQAMADQYILHLMNLTEEQRNAFRQSLSDDPSVSMIVLYKADWLNDKQAPKIAAKFDEAQSAADSEILHLPNLTEEQRNAFRQSLSDDPSVSLEVLGEAQKLNDSQAPK

SEQ ID NO: 19 - protein, 174 aa, Artificial Sequence
  fusion protein CID206137 (SEQ ID NO: 6 with PAdelFc)
IAAKFDEAQSAADSEILHLPNLTEEQRNAFRQSLSDDPSVSLEVLGEAQKLNDSQAPKIAAKFDDIQMMADAQILILYNLTEEQRNAFRQSLSDDPSVSLVVLYKADWLNRHQAPKIAAKFDEAQSAADSEILHLPNLTEEQRNAFRQSLSDDPSVSLEVLGEAQKLNDSQAPK

SEQ ID NO: 20 - protein, 174 aa, Artificial Sequence
  fusion protein CID206141 (SEQ ID NO: 5 with PAdelFc)
IAAKFDEAQSAADSEILHLPNLTEEQRNAFRQSLSDDPSVSLEVLGEAQKLNDSQAPKIAAKFDYIQEMADKHILMLHNLTEEQRNAFRQSLSDDPSVSMLVLYKAHWLNQSQAPKIAAKFDEAQSAADSEILHLPNLTEEQRNAFRQSLSDDPSVSLEVLGEAQKLNDSQAPK

SEQ ID NO: 21 - protein, 174 aa, Artificial Sequence
  fusion protein CID206142 (SEQ ID NO: 4 with PAdelFc)
IAAKFDEAQSAADSEILHLPNLTEEQRNAFRQSLSDDPSVSLEVLGEAQKLNDSQAPKIAAKFDYIQHMADDYILQLRNLTEEQRNAFRQSLSDDPSVSMVVLYRADWLNEHQAPKIAAKFDEAQSAADSEILHLPNLTEEQRNAFRQSLSDDPSVSLEVLGEAQKLNDSQAPK

SEQ ID NO: 22 - protein, 174 aa, Artificial Sequence
  fusion protein CID206146 (SEQ ID NO: 3 with PAdelFc)
IAAKFDEAQSAADSEILHLPNLTEEQRNAFRQSLSDDPSVSLEVLGEAQKLNDSQAPKIAAKFDYVQSMADAQILQLINLTEEQRNAFRQSLSDDPSVSMVVLYRADWLNEHQAPKIAAKFDEAQSAADSEILHLPNLTEEQRNAFRQSLSDDPSVSLEVLGEAQKLNDSQAPK

SEQ ID NO: 23 - protein, 185 aa, Artificial Sequence
  fusion protein CID206113 (SEQ ID NO: 9 with PAdelFc; Streptag, Cys)
IAAKFDEAQSAADSEILHLPNLTEEQRNAFRQSLSDDPSVSLEVLGEAQKLNDSQAPKNAASEDWAQFSAMYEIDHLPNLTMRQAIWFIHSLYHDPSVSKEVLGEAQKLNDSQAPKIAAKFDEAQSAADSEILHLPNLTEEQRNAFRQSLSDDPSVSLEVLGEAQKLNDSQAPKCSAWSHPQFEK

SEQ ID NO: 24 - protein, 185 aa, Artificial Sequence
  fusion protein CID206121 (SEQ ID NO: 8 with PAdelFc; Streptag, Cys)
IAAKFDEAQSAADSEILHLPNLTEEQRNAFRQSLSDDPSVSLEVLGEAQKLNDSQAPKIAAKFDEAQSAADSEILHLPNLTEYHRIQHRYWLVWDPSVSQFTLRDAQALNDWQAPKIAAKFDEAQSAADSEILHLPNLTEEQRNAFRQSLSDDPSVSLEVLGEAQKLNDSQAPKCSAWSHPQFEK

SEQ ID NO: 25 - protein, 185 aa, Artificial Sequence
  fusion protein CID206136 (SEQ ID NO: 7 with PAdelFc; Streptag, Cys)
IAAKFDEAQSAADSEILHLPNLTEEQRNAFRQSLSDDPSVSLEVLGEAQKLNDSQAPKIAAKFDQIQAMADQYILHLMNLTEEQRNAFRQSLSDDPSVSMIVLYKADWLNDKQAPKIAAKFDEAQSAADSEILHLPNLTEEQRNAFRQSLSDDPSVSLEVLGEAQKLNDSQAPKCSAWSHPQFEK

SEQ ID NO: 26 - protein, 185 aa, Artificial Sequence
  fusion protein CID206137 (SEQ ID NO: 6 with PAdelFc; Streptag, Cys)
IAAKFDEAQSAADSEILHLPNLTEEQRNAFRQSLSDDPSVSLEVLGEAQKLNDSQAPKIAAKFDDIQMMADAQILILYNLTEEQRNAFRQSLSDDPSVSLVVLYKADWLNRHQAPKIAAKFDEAQSAADSEILHLPNLTEEQRNAFRQSLSDDPSVSLEVLGEAQKLNDSQAPKCSAWSHPQFEK

SEQ ID NO: 27 - protein, 185 aa, Artificial Sequence
  fusion protein CID206141 (SEQ ID NO: 5 with PAdelFc; Streptag, Cys)
IAAKFDEAQSAADSEILHLPNLTEEQRNAFRQSLSDDPSVSLEVLGEAQKLNDSQAPKIAAKFDYIQEMADKHILMLHNLTEEQRNAFRQSLSDDPSVSMLVLYKAHWLNQSQAPKIAAKFDEAQSAADSEILHLPNLTEEQRNAFRQSLSDDPSVSLEVLGEAQKLNDSQAPKCSAWSHPQFEK

SEQ ID NO: 28 - protein, 185 aa, Artificial Sequence
  fusion protein CID206142 (SEQ ID NO: 4 with PAdelFc; Streptag, Cys)
IAAKFDEAQSAADSEILHLPNLTEEQRNAFRQSLSDDPSVSLEVLGEAQKLNDSQAPKIAAKFDYIQHMADDYILQLRNLTEEQRNAFRQSLSDDPSVSMVVLYRADWLNEHQAPKIAAKFDEAQSAADSEILHLPNLTEEQRNAFRQSLSDDPSVSLEVLGEAQKLNDSQAPKCSAWSHPQFEK

SEQ ID NO: 29 - protein, 185 aa, Artificial Sequence
  fusion protein CID206146 (SEQ ID NO: 3 with PAdelFc; Streptag, Cys)
IAAKFDEAQSAADSEILHLPNLTEEQRNAFRQSLSDDPSVSLEVLGEAQKLNDSQAPKIAAKFDYVQSMADAQILQLINLTEEQRNAFRQSLSDDPSVSMVVLYRADWLNEHQAPKIAAKFDEAQSAADSEILHLPNLTEEQRNAFRQSLSDDPSVSLEVLGEAQKLNDSQAPKCSAWSHPQFEK

SEQ ID NO: 30 - protein, 58 aa, Artificial Sequence
  PAdelFc
IAAKFDEAQSAADSEILHLPNLTEEQRNAFRQSLSDDPSVSLEVLGEAQKLNDSQAPK

SEQ ID NO: 31 - protein, 806 aa, Artificial Sequence
  FGFR3 Genbank Accession number NP 000133
MGAPACALALCVAVAIVAGASSESLGTEQRVVGRAAEVPGPEPGQQEQLVFGSGDAVELSCPPPGGGPMGPTVWVKDGTGLVPSERVLVGPQRLQVLNASHEDSGAYSCRQRLTQRVLCHFSVRVTDAPSSGDDEDGEDEAEDTGVDTGAPYWTRPERMDKKLLAVPAANTVRFRCPAAGNPTPSISWLKNGREFRGEHRIGGIKLRHQQWSLVMESVVPSDRGNYTCVVENKFGSIRQTYTLDVLERSPHRPILQAGLPANQTAVLGSDVEFHCKVYSDAQPHIQWLKHVEVNGSKVGPDGTPYVTVLKTAGANTTDKELEVLSLHNVTFEDAGEYTCLAGNSIGFSHHSAWLVVLPAEEELVEADEAGSVYAGILSYGVGFFLFILVVAAVTLCRLRSPPKKGLGSPTVHKISRFPLKRQVSLESNASMSSNTPLVRIARLSSGEGPTLANVSELELPADPKWELSRARLTLGKPLGEGCFGQVVMAEAIGIDKDRAAKPVTVAVKMLKDDATDKDLSDLVSEMEMMKMIGKHKNIINLLGACTQGGPLYVLVEYAAKGNLREFLRARRPPGLDYSFDTCKPPEEQLTFKDLVSCAYQVARGMEYLASQKCIHRDLAARNVLVTEDNVMKIADFGLARDVHNLDYYKKTTNGRLPVKWMAPEALFDRVYTHQSDVWSFGVLLWEIFTLGGSPYPGIPVEELFKLLKEGHRMDKPANCTHDLYMIMRECWHAAPSQRPTFKQLVEDLDRVLTVTSTDEYLDLSAPFEQYSPGGQDTPSSSSSGDDSVFAHDLLPPAPPSSGGSRT

SEQ ID NO: 32 - protein, 352 aa, Artificial Sequence
  extracellular domain (ECD) of Genbank Accession Number NP000133 (amino acids 23-375)
SLGTEQRVVGRAAEVPGPEPGQQEQLVFGSGDAVELSCPPPGGGPMGPTVWVKDGTGLVPSERVLVGPQRLQVLNASHEDSGAYSCRQRLTQRVLCHFSVRVTDAPSSGDDEDGEDEAEDTGVDTGAPYWTRPERMDKKLLAVPAANTVRFRCPAAGNPTPSISWLKNGREFRGEHRIGGIKLRHQQWSLVMESVVPSDRGNYTCVVENKFGSIRQTYTLDVLERSPHRPILQAGLPANQTAVLGSDVEFHCKVYSDAQPHIQWLKHVEVNGSKVGPDGTPYVTVLKTAGANTTDKELEVLSLHNVTFEDAGEYTCLAGNSIGFSHHSAWLVVLPAEEELVEADEAGSVYAG

SEQ ID NO: 33 - protein, 10 aa, Artificial Sequence
  streptag
SAWSHPQFEK

SEQ ID NO: 34 - protein, 58 aa, Artificial Sequence
  C27
NAAKFDEAQQSAFYEILHLPNLTEEQRNAFIQSLKDDPSVSKEVLGEAQKLNDSQAPK

SEQ ID NO: 35 - DNA, 708 bp, Artificial Sequence
  DNA sequence 206078 (tetramer of SEQ ID NO: 1)
atgatcgcagccaaattcgatcataaacagagcaccgcagataccattattctggaactgccgaatctgaccgaagaacagcgtaatgcatttcgtcagagcctgagtgatgatccgagcgttagcaaagaagttctgtacgaagccatttggctgaattggagccaggcaccgaaaattgcagcaaaatttgaccacaaacagtcaacagccgatacaatcattttagaactgcctaacttaacagaggaacagcgcaacgcctttcgccagtcactgtcagatgatccgtcagtttcaaaagaggtgctgtacgaggcaatctggttaaattggtcacaagcccctaaaatcgctgcgaagtttgatcataagcagtctacagcggatacgataatcctggaattaccgaatttaacggaagaacaacgcaatgcgttccgccagagtctgagcgacgatccttcagtgagtaaagaagtgttatacgaggcgatatggctgaactggtcacaggctccaaaaatagccgcaaagttcgatcacaagcaatcaaccgctgacacaatcatcctggaacttccaaaccttaccgaggaacaaagaaatgccttccgtcaaagcctgtccgacgatccgagtgtgtccaaagaggttttatacgaagctatatggttaaattggagtcaagctccgaaatgctaatga

SEQ ID NO: 36 - protein, 58 aa, Artificial Sequence
  PAdelFc
IAAQHDKDQSAADSEILHLPNLTEEQRNAFRQSLSDDPSVSLEILAEAKKLNDAQAPK

SEQ ID NO: 37 - protein, 58 aa, Artificial Sequence
  PAdelFc
IAAQHDKDQQAADKEILHLPNLTEEQRNKFRQSLRDDPSVSAEILAEAKKLNDAQAPK

SEQ ID NO: 38 - DNA, 174 bp, Artificial Sequence
  nucleotide sequence coding for SEQ ID NO: 1
atcgcagccaaattcgatcataaacagagcaccgcagataccattattctggaactgccgaatctgaccgaagaacagcgtaatgcatttcgtcagagcctgagtgatgatccgagcgttagcaaagaagttctgtacgaagccatttggctgaattggagccaggcaccgaaa

SEQ ID NO: 39 - protein, 229 aa, Artificial Sequence
  Fusion protein of sFGFR3 binding protein and non-Ig binding protein (SEQ ID NO: 1 del2N - SEQ ID NO: 1 - PAdelFc2N - PAdelFc - Cys)
AKFDHKQSTADTIILELPNLTEEQRNAFRQSLSDDPSVSKEVLYEAIWLNWSQAPKIAAKFDHKQSTADTIILELPNLTEEQRNAFRQSLSDDPSVSKEVLYEAIWLNWSQAPKAQHDKIQQAADKEILHLPNLTEEQRNKFRQSLRDDPSVSAEILAEAKKLNDAQAPKIAAQHDKIQQAADKEILHLPNLTEEQRNKFRQSLRDDPSVSAEILAEAKKLNDAQAPKC

SEQ ID NO: 40 - protein, 233 aa, Artificial Sequence
  Fusion protein of sFGFR3 binding protein and non-Ig binding protein (SEQ ID NO: 1 dimer - PAdelFc dimer), CID 206079
IAAKFDHKQSTADTIILELPNLTEEQRNAFRQSLSDDPSVSKEVLYEAIWLNWSQAPKIAAKFDHKQSTADTIILELPNLTEEQRNAFRQSLSDDPSVSKEVLYEAIWLNWSQAPKIAAKFDEAQQAADYEILHLPNLTEEQRNAFRQSLRDDPSVSLEVLGEAQKLNDSQAPKIAAKFDEAQQAADYEILHLPNLTEEQRNAFRQSLRDDPSVSLEVLGEAQKLNDSQAPKC

SEQ ID NO: 41 - protein, 229 aa, Artificial Sequence
  Fusion protein of sFGFR3 binding protein and non-Ig binding protein (SEQ ID NO: 2 del2N - SEQ ID NO: 2 - PAdelFc2N - PAdelFc - Cys)
AKFDQHQSTADEIILKLPNLTEEQRNAFRQSLSDDTSVSREVLYEALWLNASQAPKIAAKFDQHQSTADEIILKLPNLTEEQRNAFRQSLSDDTSVSREVLYEALWLNASQAPKAQHDKIQQAADKEILHLPNLTEEQRNKFRQSLRDDPSVSAEILAEAKKLNDAQAPKIAAQHDKIQQAADKEILHLPNLTEEQRNKFRQSLRDDPSVSAEILAEAKKLNDAQAPKC

SEQ ID NO: 42 - protein, 233 aa, Artificial Sequence
  Fusion protein of sFGFR3 binding protein and non-Ig binding protein (SEQ ID NO: 2 dimer - PAdelFc dimer - Cys)
IAAKFDQHQSTADEIILKLPNLTEEQRNAFRQSLSDDTSVSREVLYEALWLNASQAPKIAAKFDQHQSTADEIILKLPNLTEEQRNAFRQSLSDDTSVSREVLYEALWLNASQAPKIAAKFDEAQQAADYEILHLPNLTEEQRNAFRQSLRDDPSVSLEVLGEAQKLNDSQAPKIAAKFDEAQQAADYEILHLPNLTEEQRNAFRQSLRDDPSVSLEVLGEAQKLNDSQAPKC

SEQ ID NO: 43 - protein, 233 aa, Artificial Sequence
  Fusion protein PAdelFc-SEQ1-SEQ1-PAdelFc; CID 206080
IAAKFDEAQQAADYEILHLPNLTEEQRNAFRQSLRDDPSVSLEVLGEAQKLNDSQAPKIAAKFDHKQSTADTIILELPNLTEEQRNAFRQSLSDDPSVSKEVLYEAIWLNWSQAPKIAAKFDHKQSTADTIILELPNLTEEQRNAFRQSLSDDPSVSKEVLYEAIWLNWSQAPKIAAKFDEAQQAADYEILHLPNLTEEQRNAFRQSLRDDPSVSLEVLGEAQKLNDSQAPKC

SEQ ID NO: 44 - protein, 233 aa, Artificial Sequence
  fusion protein of SEQ ID NO: 1 - SEQ ID NO: 2- PAdelFc-PAdelFc; CID206081
IAAKFDHKQSTADTIILELPNLTEEQRNAFRQSLSDDPSVSKEVLYEAIWLNWSQAPKIAAKFDQHQSTADEIILKLPNLTEEQRNAFRQSLSDDTSVSREVLYEALWLNASQAPKIAAKFDEAQQAADYEILHLPNLTEEQRNAFRQSLRDDPSVSLEVLGEAQKLNDSQAPKIAAKFDEAQQAADYEILHLPNLTEEQRNAFRQSLRDDPSVSLEVLGEAQKLNDSQAPKC

SEQ ID NO: 45 - protein, 233 aa, Artificial Sequence
  fusion protein of SEQ ID NO: 1 - PAdelFc - SEQ ID NO: 2- PAdelFc; CID206082
IAAKFDHKQSTADTIILELPNLTEEQRNAFRQSLSDDPSVSKEVLYEAIWLNWSQAPKIAAKFDEAQQAADYEILHLPNLTEEQRNAFRQSLRDDPSVSLEVLGEAQKLNDSQAPKIAAKFDQHQSTADEIILKLPNLTEEQRNAFRQSLSDDTSVSREVLYEALWLNASQAPKIAAKFDEAQQAADYEILHLPNLTEEQRNAFRQSLRDDPSVSLEVLGEAQKLNDSQAPKC

SEQ ID NO: 46 - protein, 233 aa, Artificial Sequence
  fusion protein of SEQ ID NO: 2 - PAdelFc - SEQ ID NO: 1 - PAdelFc; CID206083
IAAKFDQHQSTADEIILKLPNLTEEQRNAFRQSLSDDTSVSREVLYEALWLNASQAPKIAAKFDEAQQAADYEILHLPNLTEEQRNAFRQSLRDDPSVSLEVLGEAQKLNDSQAPKIAAKFDHKQSTADTIILELPNLTEEQRNAFRQSLSDDPSVSKEVLYEAIWLNWSQAPKIAAKFDEAQQAADYEILHLPNLTEEQRNAFRQSLRDDPSVSLEVLGEAQKLNDSQAPKC

SEQ ID NO: 47 - protein, 56 aa, Artificial Sequence
  sFGFR3 binding protein (204815 delN2)
AKFDHKQSTADTIILELPNLTEEQRNAFRQSLSDDPSVSKEVLYEAIWLNWSQAPK

SEQ ID NO: 48 - protein, 56 aa, Artificial Sequence
  sFGFR3 bindng protein (204783 delN2)
AKFDQHQSTADEIILKLPNLTEEQRNAFRQSLSDDTSVSREVLYEALWLNASQAPK